European Patent Specification EP 3 442 566 B1, published January 21, 2026. Title: INHIBITION OF SCUBE2, A NOVEL VEGFR2 CO-RECEPTOR, SUPPRESSES TUMOR ANGIOGENESIS. Applicant: ACADEMIA SINICA. The sequence listing filed with the application follows.

SEQUENCE LISTING (102 sequences)

SEQ ID NO: 1 - protein, 119 aa, Artificial Sequence
  mAb EGF-C3 VH  domain
EVKLVESGGGLVQPGGSRKLSCVASGFTISSFGMHWVRQAPERGLEWVAYISSGSNTIYYADTVKGRFTISRDNPKNTLFLQMTSLWSEDTAMYYCARSGTLDGWFTYWGRGTLVTVST

SEQ ID NO: 2 - protein, 112 aa, Artificial Sequence
  mAb EGF-C3 VL domain
DIVMTQPPLSLPVSLGDQASISCRSSQSILHSNGNTYLEWYLQKPGQSPKLLIYKLFNRFSGVPDRFNGSGSGTDFTLKISRAEAEDLGVYYCLQGSHVPPTFGAGTKLEIK

SEQ ID NO: 3 - protein, 10 aa, Artificial Sequence
  mAb EGF-C3 VH  CDR1
GFTISSFGMH

SEQ ID NO: 4 - protein, 17 aa, Artificial Sequence
  mAb EGF-C3 VH  CDR2
YISSGSNTIYYADTVKG

SEQ ID NO: 5 - protein, 10 aa, Artificial Sequence
  mAb EGF-C3 VH CDR3
SGTLDGWFTY

SEQ ID NO: 6 - protein, 16 aa, Artificial Sequence
  mAb EGF-C3 VL  CDR1
RSSQSILHSNGNTYLE

SEQ ID NO: 7 - protein, 7 aa, Artificial Sequence
  mAb EGF-C3 VL CDR2
KLFNRFS

SEQ ID NO: 8 - protein, 9 aa, Artificial Sequence
  mAb EGF-C3 VL CDR3
LQGSHVPPT

SEQ ID NO: 9 - protein, 25 aa, Artificial Sequence
  mAb EGF-C3 VH FW1
EVKLVESGGGLVQPGGSRKLSCVAS

SEQ ID NO: 10 - protein, 14 aa, Artificial Sequence
  mAb EGF-C3 VH FW2
WVRQAPERGLEWVA

SEQ ID NO: 11 - protein, 32 aa, Artificial Sequence
  mAb EGF-C3 VH FW3
RFTISRDNPKNTLFLQMTSLWSEDTAMYYCAR

SEQ ID NO: 12 - protein, 11 aa, Artificial Sequence
  mAb EGF-C3 VH  FW4
WGRGTLVTVST

SEQ ID NO: 13 - protein, 23 aa, Artificial Sequence
  mAb EGF-C3 VL  FW1
DIVMTQPPLSLPVSLGDQASISC

SEQ ID NO: 14 - protein, 15 aa, Artificial Sequence
  mAb EGF-C3 VL FW2
WYLQKPGQSPKLLIY

SEQ ID NO: 15 - protein, 32 aa, Artificial Sequence
  mAb EGF-C3 VL  FW3
GVPDRFNGSGSGTDFTLKISRAEAEDLGVYYC

SEQ ID NO: 16 - protein, 10 aa, Artificial Sequence
  mAb EGF-C3 VL FW4
FGAGTKLEIK

SEQ ID NO: 17 - protein, 119 aa, Artificial Sequence
  mAb SP-A1 /B1 VH  domain
EVQLQQSGPELVKPGASVKVSCKASGYAFTSYNMYWVKQSHGKSLEWIGYIDPYNGDTNNNQKFKGKATLTVDKSSSTAYMHLNSLTSEDSAVYYCARSYRYLAWFAYWGQGTLVTVSA

SEQ ID NO: 18 - protein, 112 aa, Artificial Sequence
  mAb SP-A1 /B1 VL  domain
DIVMTQSPLSLPVSLGDQASISCRSSQSIVHSNGNTYLEWYLQKPGQSPKLLIYTVSNRFSGVPDRFSGSGSGTDFTLRISRVEAEDLGVYYCFQGSHIPYTFGGGTKLELK

SEQ ID NO: 19 - protein, 10 aa, Artificial Sequence
  mAb SP-A1/B1 VH CDR1
GYAFTSYNMY

SEQ ID NO: 20 - protein, 17 aa, Artificial Sequence
  mAb SP-A1/B1 VH CDR2
YIDPYNGDTNNNQKFKG

SEQ ID NO: 21 - protein, 10 aa, Artificial Sequence
  mAb SP-A1/B1 VH  CDR3
SYRYLAWFAY

SEQ ID NO: 22 - protein, 16 aa, Artificial Sequence
  mAb SP-A1/B1VL  CDR1
RSSQSIVHSNGNTYLE

SEQ ID NO: 23 - protein, 7 aa, Artificial Sequence
  mAb SP-A1/B1 VL  CDR2
TVSNRFS

SEQ ID NO: 24 - protein, 9 aa, Artificial Sequence
  mAb SP-A1/B1 VL  CDR3
FQGSHIPYT

SEQ ID NO: 25 - protein, 25 aa, Artificial Sequence
  mAb SP-A1/B1 VH  FW1
EVQLQQSGPELVKPGASVKVSCKAS

SEQ ID NO: 26 - protein, 14 aa, Artificial Sequence
  mAb SP-A1/B1 VH  FW2
WVKQSHGKSLEWIG

SEQ ID NO: 27 - protein, 32 aa, Artificial Sequence
  mAb SP-A1/B1 VH  FW3
KATLTVDKSSSTAYMHLNSLTSEDSAVYYCAR

SEQ ID NO: 28 - protein, 11 aa, Artificial Sequence
  mAb SP-A1/B1 VH  FW4
WGQGTLVTVSA

SEQ ID NO: 29 - protein, 23 aa, Artificial Sequence
  mAb SP-A1/B1 VL  FW1
DIVMTQSPLSLPVSLGDQASISC

SEQ ID NO: 30 - protein, 15 aa, Artificial Sequence
  mAb SP-A1/B1 VL  FW2
WYLQKPGQSPKLLIY

SEQ ID NO: 31 - protein, 32 aa, Artificial Sequence
  mAb SP-A1/B1 VL  FW3
GVPDRFSGSGSGTDFTLRISRVEAEDLGVYYC

SEQ ID NO: 32 - protein, 10 aa, Artificial Sequence
  mAb SP-A1/B1 VL  FW4
FGGGTKLELK

SEQ ID NO: 33 - protein, 122 aa, Artificial Sequence
  mAb SP-B2 VH  domain
EVQRVESGGGLVKPGGSLKLSCAASGFTFRNYAMSWVRQTTEKKLEWVATINDVGSYTYFPASVKGRFTVSRDNTKNTLYLQMSSLRSEDTAMYYCVTSSDTVPHHHALDYWGQGSSVTVSS

SEQ ID NO: 34 - protein, 110 aa, Artificial Sequence
  mAb SP-B2 VL  domain
DIVMTQPPASLAVSLGQRATVFCRASQNVDSRGISFMHWYQQKPGQPPKLLIYAASNLESGIPARFRGSGSGTDFTLNIHPVEEEDVATYYCQQSVEDLTFGGGTKLELK

SEQ ID NO: 35 - protein, 10 aa, Artificial Sequence
  mAb SP-B2 VH  CDR1
GFTFRNYAMS

SEQ ID NO: 36 - protein, 17 aa, Artificial Sequence
  mAb SP-B2 VH  CDR2
TINDVGSYTYFPASVKG

SEQ ID NO: 37 - protein, 13 aa, Artificial Sequence
  mAb SP-B2 VH  CDR3
SSDTVPHHHALDY

SEQ ID NO: 38 - protein, 15 aa, Artificial Sequence
  mAb SP-B2 VL CDR1
RASQNVDSRGISFMH

SEQ ID NO: 39 - protein, 7 aa, Artificial Sequence
  mAb SP-B2 VL CDR2
AASNLES

SEQ ID NO: 40 - protein, 8 aa, Artificial Sequence
  mAb SP-B2 VL CDR3
QQSVEDLT

SEQ ID NO: 41 - protein, 25 aa, Artificial Sequence
  mAb SP-B2 VH  FW1
EVQRVESGGGLVKPGGSLKLSCAAS

SEQ ID NO: 42 - protein, 14 aa, Artificial Sequence
  mAb SP-B2 VH  FW2
WVRQTTEKKLEWVA

SEQ ID NO: 43 - protein, 32 aa, Artificial Sequence
  mAb SP-B2 VH  FW3
RFTVSRDNTKNTLYLQMSSLRSEDTAMYYCVT

SEQ ID NO: 44 - protein, 11 aa, Artificial Sequence
  mAb SP-B2 VH  FW4
WGQGSSVTVSS

SEQ ID NO: 45 - protein, 23 aa, Artificial Sequence
  mAb SP-B2 VL FW1
DIVMTQPPASLAVSLGQRATVFC

SEQ ID NO: 46 - protein, 15 aa, Artificial Sequence
  mAb SP-B2 VL FW2
WYQQKPGQPPKLLIY

SEQ ID NO: 47 - protein, 32 aa, Artificial Sequence
  mAb SP-B2 VL  FW3
GIPARFRGSGSGTDFTLNIHPVEEEDVATYYC

SEQ ID NO: 48 - protein, 10 aa, Artificial Sequence
  mAb SP-B2 VL FW4
FGGGTKLELK

SEQ ID NO: 49 - protein, 120 aa, Artificial Sequence
  mAb CR-#5 VH  domain
EVQRVESGGDLVKPGGTLKLSCAASGFTFRNYGMSWVRQTPDKRLEWVATISSGGVYIYYPDSVKGRFTISRDNAKNTLFLQMSSLRSEDSAMYYCARDDYDGRGYFDYWGQGTTLTVSS

SEQ ID NO: 50 - protein, 112 aa, Artificial Sequence
  mAb CR-#5 VL  domain
DIVMSQSPSSLAVSAGEKVTMSCKSSQSLLNSRTRKNYLAWYQQKPGQSPKLLIYWASTRESGVPDRFTGSGSGTDFTLTISSVQAEDLAVYYCKQSYNLPTFGSGTKLDIK

SEQ ID NO: 51 - protein, 10 aa, Artificial Sequence
  mAb CR-#5 VH CDR1
GFTFRNYGMS

SEQ ID NO: 52 - protein, 17 aa, Artificial Sequence
  mAb CR-#5 VH  CDR2
TISSGGVYIYYPDSVKG

SEQ ID NO: 53 - protein, 13 aa, Artificial Sequence
  mAb CR-#5 VH  CDR3
ARDDYDGRGYFDY

SEQ ID NO: 54 - protein, 17 aa, Artificial Sequence
  mAb CR-#5 VL  CDR1
KSSQSLLNSRTRKNYLA

SEQ ID NO: 55 - protein, 7 aa, Artificial Sequence
  mAb CR-#5 VL  CDR2
WASTRES

SEQ ID NO: 56 - protein, 8 aa, Artificial Sequence
  mAb CR-#5 VL  CDR3
KQSYNLPT

SEQ ID NO: 57 - protein, 25 aa, Artificial Sequence
  mAb CR-#5 VH  FW1
EVQRVESGGDLVKPGGTLKLSCAAS

SEQ ID NO: 58 - protein, 14 aa, Artificial Sequence
  mAb CR-#5 VH  FW2
WVRQTPDKRLEWVA

SEQ ID NO: 59 - protein, 30 aa, Artificial Sequence
  mAb CR-#5 VH  FW3
RFTISRDNAKNTLFLQMSSLRSEDSAMYYC

SEQ ID NO: 60 - protein, 11 aa, Artificial Sequence
  mAb CR-#5 VH  FW4
WGQGTTLTVSS

SEQ ID NO: 61 - protein, 23 aa, Artificial Sequence
  mAb CR-#5 VL  FW1
DIVMSQSPSSLAVSAGEKVTMSC

SEQ ID NO: 62 - protein, 15 aa, Artificial Sequence
  mAb CR-#5 VL  FW2
WYQQKPGQSPKLLIY

SEQ ID NO: 63 - protein, 32 aa, Artificial Sequence
  mAb CR-#5 VL  FW3
GVPDRFTGSGSGTDFTLTISSVQAEDLAVYYC

SEQ ID NO: 64 - protein, 10 aa, Artificial Sequence
  mAb CR-#5 VL  FW4
FGSGTKLDIK

SEQ ID NO: 65 - DNA, 3086 bp, Artificial Sequence
  SCUBE2 cDNA
atgggggtcgcgggccgcaaccgtcccggggcggcctgggcggtgctgctgctgctgctgctgctgccgccactgctgctgctggcgggggccgtcccgccgggtcggggccgtgccgcggggccgcaggaggatgtagatgagtgtgcccaagggctagatgactgccatgccgacgccctgtgtcagaacacacccacctcctacaagtgctcctgcaagcctggctaccaaggggaaggcaggcagtgtgaggacatcgatgaatgtggaaatgagctcaatggaggctgtgtccatgactgtttgaatattccaggcaattatcgttgcacttgttttgatggcttcatgttggctcatgacggtcataattgtcttgatgtggacgagtgcctggagaacaatggcggctgccagcatacctgtgtcaacgtcatggggagctatgagtgctgctgcaaggaggggtttttcctgagtgacaatcagcacacctgcattcaccgctcggaagagggcctgagctgcatgaataaggatcacggctgtagtcacatctgcaaggaggccccaaggggcagcgtcgcctgtgagtgcaggcctggttttgagctggccaagaaccagagagactgcatcttgacctgtaaccatgggaacggtgggtgccagcactcctgtgacgatacagccgatggcccagagtgcagctgccatccacagtacaagatgcacacagatgggaggagctgccttgagcgagaggacactgtcctggaggtgacagagagcaacaccacatcagtggtggatggggataaacgggtgaaacggcggctgctcatggaaacgtgtgctgtcaacaatggaggctgtgaccgcacctgtaaggatacttcgacaggtgtccactgcagttgtcctgttggattcactctccagttggatgggaagacatgtaaagatattgatgagtgccagacccgcaatggaggttgtgatcatttctgcaaaaacatcgtgggcagttttgactgcggctgcaagaaaggatttaaattattaacagatgagaagtcttgccaagatgtggatgagtgctctttggataggacctgtgaccacagctgcatcaaccaccctggcacatttgcttgtgcttgcaaccgagggtacaccctgtatggcttcacccactgtggagacaccaatgagtgcagcatcaacaacggaggctgtcagcaggtctgtgtgaacacagtgggcagctatgaatgccagtgccaccctgggtacaagctccactggaataaaaaagactgtgtggaagtgaaggggctcctgcccacaagtgtgtcaccccgtgtgtccctgcactgcggtaagagtggtggaggagacgggtgcttcctcagatgtcactctggcattcacctctcttcaggactgcaaggggcctactctgtcacctgtggctcttcctctcctctcaggaacaaacaacaaaaatcaaatgactctgcttttggggatgtcaccaccatcaggacaagtgtaacctttaagctaaatgaaggcaagtgtagtttgaaaaatgctgagctgtttcccgagggtctgcgaccagcactaccagagaagcacagctcagtaaaagagagcttccgctacgtaaaccttacatgcagctctggcaagcaagtcccaggagcccctggccgaccaagcacccctaaggaaatgtttatcactgttgagtttgagcttgaaactaaccaaaaggaggtgacagcttcttgtgacctgagctgcatcgtaaagcgaaccgagaagcggctccgtaaagccatccgcacgctcagaaaggccgtccacagggagcagtttcacctccagctctcaggcatgaacctcgacgtggctaaaaagcctcccagaacatctgaacgccaggcagagtcctgtggagtgggccagggtcatgcagaaaaccaatgtgtcagttgcagggctgggacctattatgatggagcacgagaacgctgcattttatgtccaaatggaaccttccaaaatgaggaaggacaaatgacttgtgaaccatgcccaagaccaggaaattctggggccctgaagaccccagaagcttggaatatgtctgaatgtggaggtctgtgtcaacctggtgaatattctgcagatggctttgcaccttgccagctctgtgccctgggcacgttccagcctgaagctggtcgaacttcctgcttcccctgtggaggaggccttgccaccaaacatcagggagctacttcctttcaggactgtgaaaccagagttcaatgttcacctggacatttctacaacaccaccactcaccgatgtattcgttgcccagtgggaacataccagcctgaatttggaaaaaataattgtgtttcttgcccaggaaatactacgactgactttgatggctccacaaacataacccagtgtaaaaacagaagatgtggaggggagctgggagatttcactgggtacattgaatccccaaactacccaggcaattacccagccaacaccgagtgtacgtggaccatcaacccaccccccaagcgccgcatcctgatcgtggtccctgagatcttcctgcccatagaggacgactgtggggactatctggtgatgcggaaaacctcttctccaattctgtgacaacatatgaaacctgccagacctacgaacgccccatcgccttcacctccaggtcaaagaagctgtggattcagttcaagtccaatgaagggaacagcgctagagggttccaggtcccatacgtgacatatgatgaggactaccaggaactcattgaagacatagttcgagatggcaggctctatgcatctgagaaccatcaggaaatacttaaggataagaaacttatcaaggctctgtttgatgtcctggcccatccccagaactatttcaagtacacagcccaggagtcccgagagatgtttccaagatcgttcatccgattgctacgttccaaagtgtccaggtttttgagaccttacaaatga

SEQ ID NO: 66 - protein, 1028 aa, Homo sapiens
MGVAGRNRPGAAWAVLLLLLLLPPLLLLAGAVPPGRGRAAGPQEDVDECAQGLDDCHADALCQNTPTSYKCSCKPGYQGEGRQCEDIDECGNELNGGCVHDCLNIPGNYRCTCFDGFMLAHDGHNCLDVDECLENNGGCQHTCVNVMGSYECCCKEGFFLSDNQHTCIHRSEEGLSCMNKDHGCSHICKEAPRGSVACECRPGFELAKNQRDCILTCNHGNGGCQHSCDDTADGPECSCHPQYKMHTDGRSCLEREDTVLEVTESNTTSVVDGDKRVKRRLLMETCAVNNGGCDRTCKDTSTGVHCSCPVGFTLQLDGKTCKDIDECQTRNGGCDHFCKNIVGSFDCGCKKGFKLLTDEKSCQDVDECSLDRTCDHSCINHPGTFACACNRGYTLYGFTHCGDTNECSINNGGCQQVCVNTVGSYECQCHPGYKLHWNKKDCVEVKGLLPTSVSPRVSLHCGKSGGGDGCFLRCHSGIHLSSGLQGAYSVTCGSSSPLRNKQQKSNDSAFGDVTTIRTSVTFKLNEGKCSLKNAELFPEGLRPALPEKHSSVKESFRYVNLTCSSGKQVPGAPGRPSTPKEMFITVEFELETNQKEVTASCDLSCIVKRTEKRLRKAIRTLRKAVHREQFHLQLSGMNLDVAKKPPRTSERQAESCGVGQGHAENQCVSCRAGTYYDGARERCILCPNGTFQNEEGQMTCEPCPRPGNSGALKTPEAWNMSECGGLCQPGEYSADGFAPCQLCALGTFQPEAGRTSCFPCGGGLATKHQGATSFQDCETRVQCSPGHFYNTTTHRCIRCPVGTYQPEFGKNNCVSCPGNTTTDFDGSTNITQCKNRRCGGELGDFTGYIESPNYPGNYPANTECTWTINPPPKRRILIVVPEIFLPIEDDCGDYLVMRKTSSSNSVTTYETCQTYERPIAFTSRSKKLWIQFKSNEGNSARGFQVPYVTYDEDYQELIEDIVRDGRLYASENHQEILKDKKLIKALFDVLAHPQNYFKYTAQESREMFPRSFIRLLRSKVSRFLRPYK

SEQ ID NO: 67 - DNA, 27 bp, Artificial Sequence
  VEGF cDNA Forward primer
ccgctcgaggcacccatggcagaagga

SEQ ID NO: 68 - DNA, 32 bp, Artificial Sequence
  VEGF cDNA Reverse primer
gctctagattatcaccgcctcggcttgtcaca

SEQ ID NO: 69 - DNA, 21 bp, Artificial Sequence
  SCUBE1 Forward
tgcggcggcgagcttggtgac

SEQ ID NO: 70 - DNA, 24 bp, Artificial Sequence
  SCUBE1 Reverse
tttggagcgcagcagtttgatgaa

SEQ ID NO: 71 - DNA, 24 bp, Artificial Sequence
  SCUBE2 Forward
tcttgcccaggaaatactacgact

SEQ ID NO: 72 - DNA, 22 bp, Artificial Sequence
  SCUBE2 Reverse
tgggccaggacatcaaacagag

SEQ ID NO: 73 - DNA, 24 bp, Artificial Sequence
  SCUBE3 Forward
tggcccaatgcaagaatcgtcagt

SEQ ID NO: 74 - DNA, 21 bp, Artificial Sequence
  SCUBE3 Reverse
tgggctagcacctcaaagaag

SEQ ID NO: 75 - DNA, 20 bp, Artificial Sequence
  GAPDH Forward
gccaaaagggtcatcatctc

SEQ ID NO: 76 - DNA, 20 bp, Artificial Sequence
  GAPDH Reverse
accacctggtgctcagtgta

SEQ ID NO: 77 - DNA, 23 bp, Artificial Sequence
  mouse Scube1 Forward
cggcggcgaacttggtgactaca

SEQ ID NO: 78 - DNA, 23 bp, Artificial Sequence
  mouse Scube1 Reverse
ttgataaaggaccgggggaacat

SEQ ID NO: 79 - DNA, 24 bp, Artificial Sequence
  mouse Scube2 Forward
tgactacctggtgatgcggaaaac

SEQ ID NO: 80 - DNA, 22 bp, Artificial Sequence
  mouse Scube2 Reverse
cagtggcgtgtgggaagagtca

SEQ ID NO: 81 - DNA, 21 bp, Artificial Sequence
  mouse Scube3 Forward
tgctccccgggccactactat

SEQ ID NO: 82 - DNA, 24 bp, Artificial Sequence
  mouse Scube3 Reverse
agcgctgttggcctcactggtctt

SEQ ID NO: 83 - DNA, 21 bp, Artificial Sequence
  SCUBE2 Forward
gcacacgcacgcgcgcacaca

SEQ ID NO: 84 - DNA, 21 bp, Artificial Sequence
  SCUBE2 Reverse
gaagggtgcagagggtgtgct

SEQ ID NO: 85 - DNA, 25 bp, Artificial Sequence
  mouse Gapdh Forward
atcatccctgcatccactggtgctg

SEQ ID NO: 86 - DNA, 25 bp, Artificial Sequence
  mouse Gapdh Reverse
tgatggcattcaagagagtagggag

SEQ ID NO: 87 - DNA, 20 bp, Artificial Sequence
  SCUBE1 Forward
aacatcccggggaactacag

SEQ ID NO: 88 - DNA, 20 bp, Artificial Sequence
  SCUBE1 Reverse
gcagccaccattattgtcct

SEQ ID NO: 89 - DNA, 20 bp, Artificial Sequence
  SCUBE2 Forward
caggcagagtcctgtggagt

SEQ ID NO: 90 - DNA, 20 bp, Artificial Sequence
  SCUBE2 Reverse
taaaatgcagcgttctcgtg

SEQ ID NO: 91 - DNA, 18 bp, Artificial Sequence
  SCUBE3 Forward
cctgcttgtcctgctggt

SEQ ID NO: 92 - DNA, 20 bp, Artificial Sequence
  SCUBE3 Reverse
tcgatgtggcagttgtcagt

SEQ ID NO: 93 - DNA, 19 bp, Artificial Sequence
  GAPDH Forward
tgaaggtcggagtcaacgg

SEQ ID NO: 94 - DNA, 22 bp, Artificial Sequence
  GAPDH Reverse
agagttaaaagcagccctggtg

SEQ ID NO: 95 - DNA, 29 bp, Artificial Sequence
  Scube2-5'Flox F1
atagtcgactgttgtccagtatctgttgc

SEQ ID NO: 96 - DNA, 31 bp, Artificial Sequence
  Scube2-5'Flox R1
atagcggccgctacgacaccctgggataaag

SEQ ID NO: 97 - DNA, 23 bp, Artificial Sequence
  Scube2-3'Flox F2
ggccatgtccctgaagaaaacta

SEQ ID NO: 98 - DNA, 22 bp, Artificial Sequence
  Scube2-3'Flox R2
ttatggggccaagacactcaaa

SEQ ID NO: 99 - DNA, 22 bp, Artificial Sequence
  Scube2-Null F3
ctggggcctctgggacactatt

SEQ ID NO: 100 - DNA, 23 bp, Artificial Sequence
  Scube2-Null R3
gttatggggccaagacactcaaa

SEQ ID NO: 101 - DNA, 25 bp, Artificial Sequence
  Cre Forward
ttaccggtcgatgcaacgagtgatg

SEQ ID NO: 102 - DNA, 23 bp, Artificial Sequence
  Cre Reverse
gtgaaacagcattgctgtcactt